European Patent Application EP 4 736 866 A1, published May 6, 2026. Title: STABILIZER FOR URATE OXIDASE AND PEGYLATED CONJUGATE THEREOF, AND PHARMACEUTICAL USE OF STABILIZER. Applicant: HANGZHOU GRAND BIOLOGIC PHARMACEUTICAL INC. The sequence listing filed with the application follows.

SEQUENCE LISTING (9 sequences)

SEQ ID NO: 1 - protein, 298 aa, synthetic construct
TYKKNDEVEFVRTGYGKDMIKVLHIQRDGKYHSIKEVATTVQLTLSSKKDYLHGDNSDVIPTDTIKNTVNVLAKFKGIKSIETFAVTICEHFLSSFKHVIRAQVYVEEVPWKRFEKNGVKHVHAFIYTPTGTHFCEVEQIRNGPPVIHSGIKDLKVLKTTQSGFEGFIKDQFTTLPEVKDRCFATQVYCKWRYHQGRDVDFEATWDTVRSIVLQKFAGPYDKGEYSPSVQKTLYDIQVLTLGQVPEIEDMEISLPNIHYLNIDMSKMGLINKEEVLLPLDNPYGKITGTVKRKLSSRL

SEQ ID NO: 2 - protein, 304 aa, synthetic construct
MAHYRNDYKKNDEVEFVRTGYGKDMIKVLHIQRDGKYHSIKEVATSVQLTLSSKKDYLHGDNSDVIPTDTIKNTVNVLAKFKGIKSIETFAVTICEHFLSSFKHVIRAQVYVEEVPWKRFEKNGVKHVHAFIYTPTGTHFCEVEQIRNGPPVIHSGIKDLKVLKTTQSGFEGFIKDQFTTLPEVKDRCFATQVYCKWRYHQGRDVDFEATWDTVRSIVLQKFAGPYDKGEYSPSVQKTLYDIQVLTLGQVPEIEDMEISLPNIHYLNIDMSKMGLINKEEVLLPLDNPYGRITGTVKRKLTSRL

SEQ ID NO: 3 - protein, 297 aa, synthetic construct
MYKNDEVEFVRTGYGKDMVKVLHIQRDGKYHSIKEVATSVQLTLSSKKDYVYGDNSDIIPTDTIKNTVHVLAKFKGIKSIETFAMNICEHFLSSFNHVIRAQVYVEEVPWKRFEKNGVKHVHAFIHNPTGTHFCEVEQMRSGPPVIHSGIKDLKVLKTTQSGFEGFIKDQFTTLPEVKDRCFATKVYCKWRYHQGRDVDFEATWDTVRDIVLEKFAGPYDKGEYSPSVQKTLYDIQVHSLSRVPEMEDMEISLPNIHYFNIDMSKMGLINKEEVLLPLDNPYGKITGTVKRKLSSRL

SEQ ID NO: 4 - protein, 304 aa, synthetic construct
MAHYHNDYKKNDEVEFVRTGYGKDMVKVLHIQRDGKYHSIKEVATSVQLTLSSKKDYVYGDNSDIIPTDTIKNTVHVLAKFKGIKSIETFAMNICEHFLSSFNHVIRAQVYVEEVPWKRFEKNGVKHVHAFIHNPTGTHFCEVEQMRSGPPVIHSGIKDLKVLKTTQSGFEGFIKDQFTTLPEVKDRCFATKVYCKWRYHQGRDVDFEATWDTVRDIVLEKFAGPYDKGEYSPSVQKTLYDIQVHSLSRVPEMEDMEISLPNIHYFNIDMSKMGLINKEEVLLPLDNPYGRITGTAKRKLASKL

SEQ ID NO: 5 - protein, 304 aa, synthetic construct
MAHYHNDYQKNDEVEFVRTGYGKDMVKVLHIQRDGKYHSIKEVATSVQLTLNSRREYLHGDNSDIIPTDTIKNTVQVLAKFKGIKSIETFAMNICEHFLSSFNHVIRVQVYVEEVPWKRFEKNGVKHVHAFIHTPTGTHFCEVEQLRSGPPVIHSGIKDLKVLKTTQSGFEGFLKDQFTTLPEVKDRCFATQVYCKWRYHQGRDVDFEATWEAVRGIVLKKFAGPYDKGEYSPSVQKTLYDIQVLSLSQLPEIEDMEISLPNIHYFNIDMSKMGLINKEEVLLPLDNPYGRITGTVKRKLTSRL

SEQ ID NO: 6 - protein, 304 aa, synthetic construct
MAHYHNDYKKNDEVEFVRTGYGKDMVKVLHIQRDGKYHSIKEVATSVQLTLSSKKDYLHGDNSDIIPTDTIKNTVHALAKFKGIKSIEAFAVNICQHFLSSFNHVIRTQVYVEEIPWKRLEKNGVKHVHAFIHTPTGTHFCEVEQLRSGPPVIHSGIKDLKVLKTTQSGFEGFIKDQFTTLPEVKDRCFAAQVYCKWRYHQCRDVDFEATWDTIRDVVLEKFAGPYDKGEYSPSVQKTLYDIQVVSLSQVPEIDDMEISLPNIHYFNIDMSKMGLINKEEVLLPLDNPYGKITGTVKRKLSSRL

SEQ ID NO: 7 - protein, 304 aa, synthetic construct
MADYHNNYKKNDELEFVRTGYGKDMVKVLHIQRDGKYHSIKEVATSVQLTLSSKKDYLHGDNSDIIPTDTIKNTVHVLAKFKGIKSIEAFGVNICEYFLSSFNHVIRAQVYVEEIPWKRLEKNGVKHVHAFIHTPTGTHFCEVEQLRSGPPVIHSGIKDLKVLKTTQSGFEGFIKDQFTTLPEVKDRCFATQVYCKWRYHQCRDVDFEATWGTIRDLVLEKFAGPYDKGEYSPSVQKTLYDIQVLSLSRVPEIEDMEISLPNIHYFNIDMSKMGLINKEEVLLPLDNPYGKITGTVKRKLSSRL

SEQ ID NO: 8 - protein, 301 aa, synthetic construct
SAVKAARYGKDNVRVYKVHKDEKTGVQTVYEMTVCVLLEGEIETSYTKADNSVIVATDSIKNTIYITAKQNPVTPPELFGSILGTHFIEKYNHIHAAHVNIVCHRWTRMDIDGKPHPHSFIRDSEEKRNVQVDVVEGKGIDIKSSLSGLTVLKSTNSQFWGFLRDEYTTLKETWDRILSTDVDATWQWKNFSGLQEVRSHVPKFDATWATAREVTLKTFAEDNSASVQATMYKMAEQILARQQLIETVEYSLPNKHYFEIDLSWHKGLQNTGKNAEVFAPQSDPNGLIKCTVGRSSLKSKL

SEQ ID NO: 9 - protein, 288 aa, synthetic construct
MTNIILGKNQYGKAEVRLVKVTRNTCRHEIQDLNVTSQLRGDFEAAHTAGDNAHVVATDTQKNTVYAFARDGFATTEEFLLRLGKHFTEGFDWVTGGRWAAQQFFWDRINDHDHAFSRNKSEVRTAVLEISGSEQAIVAGIEGLTVLKSTGSEFHGFPRDKYTTLPETEDRILATDVSARWRYNTVEVDFDAVYADVRGLLLKAFAETHSLALQQTMYEMGRAVIETHPEIDEIKMSLPNKHHFLVDLSPFGQDNPNEVFYAADRPYGLIEATIQREGCRADHPIWSN